European Patent Application EP 4 545 099 A1, published April 30, 2025. Title: METHOD FOR TREATING SOLID TUMOR. Applicant: Bio-Thera Solutions, Ltd. The sequence listing filed with the application follows.

SEQUENCE LISTING (2 sequences)

SEQ ID NO: 1 - protein, 451 aa, synthetic construct
QVQLQQSGSELKKPGASVKVSCKASGYTFTNYGMNWVKQAPGQGLKWMGWINTYTGEPTYTDDFKGRFAFSLDTSVSTAYLQISSLKADDTAVYFCARGGFGSSYWYFDVWGQGTLVTVSSASTKGPSVFPLAPSSKSTSGGTAALGCLVKDYFPEPVTVSWNSGALTSGVHTFPAVLQSSGLYSLSSVVTVPSSSLGTQTYICNVNHKPSNTKVDKKVEPKSCDKTHTCPPCPAPELLGGPSVFLFPPKPKDTLMISRTPEVTCVVVDVSHEDPEVKFNWYVDGVEVHNAKTKPREEQYNSTYRVVSVLTVLHQDWLNGKEYKCKVSNKALPAPIEKTISKAKGQPREPQVYTLPPSRDELTKNQVSLTCLVKGFYPSDIAVEWESNGQPENNYKTTPPVLDSDGSFFLYSKLTVDKSRWQQGNVFSCSVMHEALHNHYTQKSLSLSPGK

SEQ ID NO: 2 - protein, 214 aa, synthetic construct
DIQLTQSPSSLSASVGDRVSITCKASQDVSIAVAWYQQKPGKAPKLLIYSASYRYTGVPDRFSGSGSGTDFTLTISSLQPEDFAVYYCQQHYITPLTFGAGTKVEIKRTVAAPSVFIFPPSDEQLKSGTASVVCLLNNFYPREAKVQWKVDNALQSGNSQESVTEQDSKDSTYSLSSTLTLSKADYEKHKVYACEVTHQGLSSPVTKSFNRGEC